European Patent Specification EP 3 682 242 B1, published March 5, 2025. Title: Verfahren zum Nachweis akuter Borna Disease Virus (BDV) Infektionen . Applicant: Ludwig, Hanns Bode, Liv. The sequence listing filed with the application follows.

SEQUENCE LISTING (10 sequences)

SEQ ID NO: 1 - protein, 370 aa, Borna Disease Virus
MPPKRRLVDDADAMEDQDLYEPPASLPKLPGKFLQYTVGGSDPHPGIGHEKDIRQNAVALLDQSRRDMFHTVTPSLVFLCLLIPGLHAAFVHGGVPRESYLSTPVTRGEQTVVKTAKFYGEKTTQRDLTELEISSIFSHCCSLLIGVVIGSSSKIKAGAEQIKKRFKTMMAALNRPSHGETATLLQMFNPHEAIDWINGQPWVGSFVLSLLTTDFESPGKEFMDQIKLVASYAQMTTYTTIKEYLAECMDATLTIPVVAYEIRDFLEVSAKLKEDHADLFPFLGAIRHPDAIKLAPRSFPNLASAAFYWSKKENPTMAGYRASTIQPGASVKETQLARYRRREISRGEDGAELSGEISAIMRMIGVTGLN

SEQ ID NO: 2 - protein, 201 aa, Borna Disease Virus
MATRPSSLVDSLEDEEDPQTLRRERSGSPRPRKVPRNALTQPVDQLLKDLRKNPSMISDPDQRTGREQLSNDELIKKLVTELAENSMIEAEEVRGTLGDISARIEAGFESLSALQVETIQTAQRCDHSDSIRILGENIKILDRSMKTMMETMKLMMEKVDLLYASTAVGTSAPMLPSHPAPPRIYPQLPSAPTTDEWDIIP

SEQ ID NO: 3 - protein, 5 aa, Borna disease Virus
KFLQY

SEQ ID NO: 4 - protein, 5 aa, borna virus disease
AKFYG

SEQ ID NO: 5 - protein, 5 aa, Borna Disease Virus
TMMAA

SEQ ID NO: 6 - protein, 5 aa, Borna Disease Virus
LAPRS

SEQ ID NO: 7 - protein, 5 aa, Borna Disease Virus
FYWSK

SEQ ID NO: 8 - protein, 15 aa, Borna Disease Virus
RRERSGSPRPRKVPR

SEQ ID NO: 9 - protein, 12 aa, Borna Disease Virus
LLKDLRKNPSMI

SEQ ID NO: 10 - protein, 5 aa, Borna Disease Virus
DRSMK